European Patent Application EP 4 477 736 A1, published December 18, 2024. Title: Genetic biocontainment system to prevent theft and misuse of biological resources and uses thereof. Applicant: POSTECH Research and Business Development Foundation. Application EP. The sequence listing filed with the application follows.

SEQUENCE LISTING (116 sequences)

SEQ ID NO: 1 - DNA, 720 bp, synthetic construct
  source 1..720: mol_type = other DNA; note = GFP
atggctagcaagggcgaggagctgttcaccggggtggtgcccatcctggtcgagctggacggcgacgtaaacggccacaagttcagcgtgcgcggcgagggcgagggcgatgccaccaacggcaagctgaccctgaagttcatctgcaccaccggcaagctgcccgtgccctggcccaccctcgtgaccaccctgacctacggcgtgcagtgcttcagccgctaccccgaccacatgaagcagcacgacttcttcaagtccgccatgcccgaaggctacgtccaggagcgcaccatcagcttcaaggacgacggcacctacaagacccgcgccgaggtgaagttcgagggcgacaccctggtgaaccgcatcgagctgaagggcatcgacttcaaggaggacggcaacatcctggggcacaagctggagtacaacttcaacagccacaacgtctatatcaccgccgacaagcagaagaacggcatcaaggccaacttcaagatccgccacaacgtggaggacggcagcgtgcagctcgccgaccactaccagcagaacacccccatcggcgacggccccgtgctgctgcccgacaaccactacctgagcacccagtccgtgctgagcaaagaccccaacgagaagcgcgatcacatggtcctgctggagttcgtgaccgccgccgggatcactctcggcatggacgagctgtacaagtaa

SEQ ID NO: 2 - DNA, 924 bp, Erwinia herbicola
  source 1..924: mol_type = genomic DNA; note = CrtE
atggtgagtggcagtaaagcgggcgtttcgcctcatcgcgaaatagaagtaatgagacaatccattgacgatcacctggctggcctgttacctgaaaccgacagccaggatatcgtcagccttgcgatgcgtgaaggcgtcatggcacccggtaaacggatccgtccgctgctgatgctgctggccgcccgcgacctccgctaccagggcagtatgcctacgctgctcgatctcgcctgcgccgttgaactgacccataccgcgtcgctgatgctcgacgacatgccctgcatggacaacgccgagctgcgccgcggtcagcccactacccacaaaaaatttggtgagagcgtggcgatccttgcctccgttgggctgctctctaaagcctttggtctgatcgccgccaccggcgatctgccgggggagaggcgtgcccaggcggtcaacgagctctctaccgccgtgggcgtgcagggcctggtactggggcagtttcgcgatcttaacgatgccgccctcgaccgtacccctgacgctatcctcagcaccaaccacctcaagaccggcattctgttcagcgcgatgctgcagatcgtcgccattgcttccgcctcgtcgccgagcacgcgagagacgctgcacgccttcgccctcgacttcggccaggcgtttcaactgctggacgatctgcgtgacgatcacccggaaaccggtaaagatcgcaataaggacgcgggaaaatcgacgctggtcaaccggctgggcgcagacgcggcccggcaaaagctgcgcgagcatattgattccgccgacaaacacctcacttttgcctgtccgcagggcggcgccatccgacagtttatgcatctgtggtttggccatcaccttgccgactggtcaccggtcatgaaaatcgcctga

SEQ ID NO: 3 - DNA, 1479 bp, Erwinia herbicola
  source 1..1479: mol_type = genomic DNA; note = Crtl
atgaaaaaaaccgttgtgattggcgcaggctttggtggcctggcgctggcgattcgcctgcaggcggcagggatcccaaccgtactgctggagcagcgggacaagcccggcggtcgggcctacgtctggcatgaccagggctttacctttgacgccgggccgacggtgatcaccgatcctaccgcgcttgaggcgctgttcaccctggccggcaggcgcatggaggattacgtcaggctgctgccggtaaaacccttctaccgactctgctgggagtccgggaagaccctcgactatgctaacgacagcgccgagcttgaggcgcagattacccagttcaacccccgcgacgtcgagggctaccggcgctttctggcttactcccaggcggtattccaggagggatatttgcgcctcggcagcgtgccgttcctctcttttcgcgacatgctgcgcgccgggccgcagctgcttaagctccaggcgtggcagagcgtctaccagtcggtttcgcgctttattgaggatgagcatctgcggcaggccttctcgttccactccctgctggtaggcggcaaccccttcaccacctcgtccatctacaccctgatccacgcccttgagcgggagtggggggtctggttccctgagggcggcaccggggcgctggtgaacggcatggtgaagctgtttaccgatctgggcggggagatcgaactcaacgcccgggtcgaagagctggtggtggccgataaccgcgtaagccaggtccggctggcggatggtcggatctttgacaccgacgccgtagcctcgaacgctgacgtggtgaacacctataaaaagctgctcggccaccatccggtggggcagaagcgggcggcagcgctggagcgcaagagcatgagcaactcgctgtttgtgctctacttcggcctgaaccagcctcattcccagctggcgcaccataccatctgttttggtccccgctaccgggagctgatcgacgagatctttaccggcagcgcgctggcggatgacttctcgctctacctgcactcgccctgcgtgaccgatccctcgctcgcgcctcccggctgcgccagcttctacgtgctggccccggtgccgcatcttggcaacgcgccgctggactgggcgcaggaggggccgaagctgcgcgaccgcatctttgactaccttgaagagcgctatatgcccggcctgcgtagccagctggtgacccagcggatctttaccccggcagacttccacgacacgctggatgcgcatctgggatcggccttctccatcgagccgctgctgacccaaagcgcctggttccgcccgcacaaccgcgacagcgacattgccaacctctacctggtgggcgcaggtactcaccctggggcgggcattcctggcgtagtggcctcggcgaaagccaccgccagcctgatgattgaggatctgcaatga

SEQ ID NO: 4 - DNA, 930 bp, Erwinia herbicola
  source 1..930: mol_type = genomic DNA; note = CrtB
atgagccaaccgccgctgcttgaccacgccacgcagaccatggccaacggctcgaaaagttttgccaccgctgcgaagctgttcgacccggccacccgccgtagcgtgctgatgctctacacctggtgccgccactgcgatgacgtcattgacgaccagacccacggcttcgccagcgaggccgcggcggaggaggaggccacccagcgcctggcccggctgcgcacgctgaccctggcggcgtttgaaggggccgagatgcaggatccggccttcgctgcctttcaggaggtggcgctgacccacggtattacgccccgcatggcgctcgatcacctcgacggctttgcgatggacgtggctcagacccgctatgtcacctttgaggatacgctgcgctactgctatcacgtggcgggcgtggtgggtctgatgatggccagggtgatgggcgtgcgggatgagcgggtgctggatcgcgcctgcgatctggggctggccttccagctgacgaatatcgcccgggatattattgacgatgcggctattgaccgctgctatctgcccgccgagtggctgcaggatgccgggctgaccccggagaactatgccgcgcgggagaatcgggccgcgctggcgcgggtggcggagcggcttattgatgccgcagagccgtactacatctcctcccaggccgggctacacgatctgccgccgcgctgcgcctgggcgatcgccaccgcccgcagcgtctaccgggagatcggtattaaggtaaaagcggcgggaggcagcgcctgggatcgccgccagcacaccagcaaaggtgaaaaaattgccatgctgatggcggcaccggggcaggttattcgggcgaagacgacgagggtgacgccgcgtccggccggtctttggcagcgtcccgtttag

SEQ ID NO: 5 - DNA, 1149 bp, synthetic construct
  source 1..1149: mol_type = other DNA; note = trfA
atgaatcggacgtttgaccggaaggcatacaggcaagaactgatcgacgcggggttttccgccgaggatgccgaaaccatcgcaagccgcaccgtcatgcgtgcgccccgcgaaaccttccagtccgtcggctcgatggtccagcaagctacggccaagatcgagcgcgacagcgtgcaactggctccccctgccctgcccgcgccatcggccgccgtggagcgttcgcgtcgtctcgaacaggaggcggcaggtttggcgaagtcgatgaccatcgacacgcgaggaactatgacgaccaagaagcgaaaaaccgccggcgaggacctggcaaaacaggtcagcgaggccaagcaggccgcgttgctgaaacacacgaagcagcagatcaaggaaatgcagctttccttgttcgatattgcgccgtggccggacacgatgcgagcgatgccaaacgacacggcccgctctgccctgttcaccacgcgcaacaagaaaatcccgcgcgaggcgctgcaaaacaaggtcattttccacgtcaacaaggacgtgaagatcacctacaccggcgtcgagctgcgggccgacgatgacgaactggtgtggcagcaggtgttggagtacgcgaagcgcacccctatcggcgagccgatcaccttcacgttctacgagctttgccaggacctgggctggtcgatcaatggccggtattacacgaaggccgaggaatgcctgtcgcgcctacaggcgacggcgatgggcttcacgtccgaccgcgttgggcacctggaatcggtgtcgctgctgcaccgcttccgcgtcctggaccgtggcaagaaaacgtcccgttgccaggtcctgatcgacgaggaaatcgtcgtgctgtttgctggcgaccactacacgaaattcatatgggagaagtaccgcaagctgtcgccgacggcccgacggatgttcgactatttcagctcgcaccgggagccgtacccgctcaagctggaaaccttccgcctcatgtgcggatcggattccacccgcgtgaagaagtggcgcgagcaggtcggcgaagcctgcgaagagttgcgaggcagcggcctggtggaacacgcctgggtcaatgatgacctggtgcattgcaaacgctag

SEQ ID NO: 6 - DNA, 1386 bp, synthetic construct
  source 1..1386: mol_type = other DNA; note = cysS
atgctaaaaatcttcaatactctgacacgccaaaaagaggaatttaagcctattcacgccggggaagtcggcatgtacgtgtgtggaatcaccgtttacgatctctgtcatatcggtcacgggcgtacctttgttgcttttgacgtggttgcgcgctatctgcgtttcctcggctataaactgaagtatgtgcgcaacattaccgatatcgacgacaaaatcatcaaacgcgccaatgaaaatggcgaaagctttgtggcgatggtggatcgcatgatcgccgaaatgcacaaagattttgatgctttgaacattctgcgcccggatatggagccgcgcgcgacgcaccatatcgcagaaattattgaactcactgaacaactgatcgccaaaggtcacgcttatgtggcggacaacggcgacgtgatgttcgacgtcccgaccgatccaacttatggcgtgctgtcgcgtcaggatctcgaccagctgcaggcaggcgcgcgcgttgacgtggtcgacgacaaacgcaacccaatggacttcgttctgtggaagatgtcgaaagagggcgaaccgagctggccgtctccgtggggcgcgggtcgtcctggctggcacattgaatgttcggcaatgaactgcaagcagctgggtaaccactttgatatccacggcggcggttcagacctgatgttcccgcaccacgaaaacgaaatcgcgcagtccacctgtgcccatgatggtcagtatgtgaactactggatgcactcggggatggtgatggttgaccgcgagaagatgtccaaatcgctgggtaacttctttaccgtgcgcgatgtgctgaaatactacgacgcggaaaccgtgcgttacttcctgatgtcgggccactatcgcagccagttgaactacagcgaagagaacctgaagcaggcgcgtgcggcgctggagcgtctctacactgcgctgcgcggcacagataaaaccgttgcgcctgccggtggcgaagcgtttgaagcgcgctttattgaagcgatggacgacgatttcaacaccccggaagcctattccgtactgtttgatatggcgcgtgaagtaaaccgtctgaaagcagaagatatggcagcggcgaatgcaatggcatctcacctgcgtaaactttccgctgtattgggcctgctggagcaagaaccggaagcgttcctgcaaagcggcgcgcaggcagacgacagcgaagtggctgagattgaagcgttaattcaacagcgtctggatgcccgtaaagcgaaagactgggcggcggcggatgcggcgcgtgatcgtcttaacgagatggggatcgtgctggaagatggcccgcaagggaccacctggcgtcgtaagtaa

SEQ ID NO: 7 - DNA, 531 bp, synthetic construct
  source 1..531: mol_type = other DNA; note = fldA
atggctatcactggcatctttttcggcagcgacaccggtaataccgaaaatatcgcaaaaatgattcaaaaacagcttggtaaagacgttgccgatgtccatgacattgcaaaaagcagcaaagaagatctggaagcttatgacattctgctgctgggcatcccaacctggtattacggcgaagcgcagtgtgactgggatgacttcttcccgactctcgaagagattgatttcaacggcaaactggttgcgctgtttggttgtggtgaccaggaagattacgccgaatatttctgcgacgcattgggcaccatccgcgacatcattgaaccgcgcggtgcaaccatcgttggtcactggccaactgcgggctatcatttcgaagcatcaaaaggtctggcagatgacgaccactttgtcggtctggctatcgacgaagaccgtcagccggaactgaccgctgaacgtgtagaaaaatgggttaaacagatttctgaagagttgcatctcgacgaaattctcaatgcctga

SEQ ID NO: 8 - DNA, 31 bp, synthetic construct
  source 1..31: mol_type = other DNA; note = Fgfp45Lmut
gacccttaagttcatctgcaccaccggcaag

SEQ ID NO: 9 - DNA, 21 bp, synthetic construct
  source 1..21: mol_type = other DNA; note = Rgfp45Lmut
agggtcagcttgccgttggtg

SEQ ID NO: 10 - DNA, 23 bp, synthetic construct
  source 1..23: mol_type = other DNA; note = Fgfp31Rmut
aggaggcgagggcgagggcgatg

SEQ ID NO: 11 - DNA, 25 bp, synthetic construct
  source 1..25: mol_type = other DNA; note = Rgfp31Rmut
cacgctgaacttgtggccgtttacg

SEQ ID NO: 12 - DNA, 90 bp, synthetic construct
  source 1..90: mol_type = other DNA; note = QargW1
gtcctcttagttaaatggatataacgagccccttcctaagggctaattgcaggttcgattcctgcaggggacaccatttatcacagattg

SEQ ID NO: 13 - DNA, 90 bp, synthetic construct
  source 1..90: mol_type = other DNA; note = QargW2
caatctgtgataaatggtgtcccctgcaggaatcgaacctgcaattagcccttaggaaggggctcgttatatccatttaactaagaggac

SEQ ID NO: 14 - DNA, 90 bp, synthetic construct
  source 1..90: mol_type = other DNA; note = QargU1
gcgcccttagctcagttggatagagcaacgaccttcctaagtcgtgggccgcaggttcgaatcctgcagggcgcgccatttatcacagat

SEQ ID NO: 15 - DNA, 90 bp, synthetic construct
  source 1..90: mol_type = other DNA; note = QargU2
atctgtgataaatggcgcgccctgcaggattcgaacctgcggcccacgacttaggaaggtcgttgctctatccaactgagctaagggcgc

SEQ ID NO: 16 - DNA, 40 bp, synthetic construct
  source 1..40: mol_type = other DNA; note = FtRNAvectorW
gcgcgccatttatcacagattggaaatttttgatccttag

SEQ ID NO: 17 - DNA, 34 bp, synthetic construct
  source 1..34: mol_type = other DNA; note = RtRNAvectorW
actgagctaagggcgcaatgcgtctgatggcagc

SEQ ID NO: 18 - DNA, 38 bp, synthetic construct
  source 1..38: mol_type = other DNA; note = FtRNAvectorU
acaccatttatcacagattggaaatttttgatccttag

SEQ ID NO: 19 - DNA, 35 bp, synthetic construct
  source 1..35: mol_type = other DNA; note = RtRNAvectorU
catttaactaagaggacaatgcgtctgatggcagc

SEQ ID NO: 20 - DNA, 23 bp, synthetic construct
  source 1..23: mol_type = other DNA; note = FpLPP
caaatgtagcacctgaagtcagc

SEQ ID NO: 21 - DNA, 33 bp, synthetic construct
  source 1..33: mol_type = other DNA; note = RrrnBTT
ccgctcgagggcatcggtcgactaaaaaaaatc

SEQ ID NO: 22 - DNA, 39 bp, synthetic construct
  source 1..39: mol_type = other DNA; note = FkmR
tctactgaaccgcggatcccatatggtcgacctgcaggc

SEQ ID NO: 23 - DNA, 30 bp, synthetic construct
  source 1..30: mol_type = other DNA; note = RkmR
cagccggatcggatctgtaatccgggcagc

SEQ ID NO: 24 - DNA, 29 bp, synthetic construct
  source 1..29: mol_type = other DNA; note = Fcdfvector
ttacagatccgatccggctgctaacaaag

SEQ ID NO: 25 - DNA, 32 bp, synthetic construct
  source 1..32: mol_type = other DNA; note = Rcdfvector
catatgggatccgcggttcagtagaaaagatc

SEQ ID NO: 26 - DNA, 29 bp, synthetic construct
  source 1..29: mol_type = other DNA; note = FQkmR
accgcgattaaattccaacatggatgctg

SEQ ID NO: 27 - DNA, 31 bp, synthetic construct
  source 1..31: mol_type = other DNA; note = RQkmR
tcctcgagcaagacgtttcccgttgaatatg

SEQ ID NO: 28 - DNA, 31 bp, synthetic construct
  source 1..31: mol_type = other DNA; note = FcrtE
gagatatacatatggtgagtggcagtaaagc

SEQ ID NO: 29 - DNA, 30 bp, synthetic construct
  source 1..30: mol_type = other DNA; note = RctrB
ccgctcgagctaaacgggacgctgccaaag

SEQ ID NO: 30 - DNA, 23 bp, synthetic construct
  source 1..23: mol_type = other DNA; note = Fptrc
tctagatttcagtgctccttgac

SEQ ID NO: 31 - DNA, 90 bp, synthetic construct
  source 1..90: mol_type = other DNA; note = MAGE_lptF
accagattcgccggaatatcgccgtcaaccgctgcgccgaggattctcactaacttttgacagaagaagatcaaaagcaagatgaagagt

SEQ ID NO: 32 - DNA, 90 bp, synthetic construct
  source 1..90: mol_type = other DNA; note = MAGE_dnaC
tcatcaccgtggccgatattatgtcggcgatgaaagataccttcagaaatagcggtaccagcgaagaacaactgcttaacgatctgagca

SEQ ID NO: 33 - DNA, 90 bp, synthetic construct
  source 1..90: mol_type = other DNA; note = MAGE_ ftsL
ttttgcactacgatattttcttgtgacggatcaacatgctgcatttgcagcttttccgtggcgattctttccacccggctatggtcgccg

SEQ ID NO: 34 - DNA, 90 bp, synthetic construct
  source 1..90: mol_type = other DNA; note = MAGE_lpxC
gtatgtaaaccgacacccgtcgcctgaacgatacgtttaagtgttctttgtttgatcatcgtattatctcgccaaattacctatccaacc

SEQ ID NO: 35 - DNA, 90 bp, synthetic construct
  source 1..90: mol_type = other DNA; note = MAGE_ispU
atttgccaaagcaaaaagttactaatgcgatgctcccccccagttctaattactaaatctacaggggccagttcatgcatacagacatgc

SEQ ID NO: 36 - DNA, 90 bp, synthetic construct
  source 1..90: mol_type = other DNA; note = MAGE_cdsA
caaatcccagagaaaactcagcatattaccttccgttaaagcgttctgaataccagtaacaacaagcaagcaaagaccggtaccgcagcc

SEQ ID NO: 37 - DNA, 90 bp, synthetic construct
  source 1..90: mol_type = other DNA; note = MAGE_rseP
aaggtcacccactgcgttaagggctgaccatcgactttaacgattctgtcgcctgcttgcaaacctgccttgcttgccgccgagtttggc

SEQ ID NO: 38 - DNA, 90 bp, synthetic construct
  source 1..90: mol_type = other DNA; note = MAGE_tilS
cgtaaacagggtgaggcatcttcccgcgccagcgccacttcctgccagattctcaccaacgcgtcgcgggaaggcatcggtgcattctgc

SEQ ID NO: 39 - DNA, 90 bp, synthetic construct
  source 1..90: mol_type = other DNA; note = MAGE_mrdB
tgctgatggctgggttcgggattgtaatgtcaatccacacccacagaaaaatgttgtcgaaaagcgtgtaagaggtgcgcaatgcgtaag

SEQ ID NO: 40 - DNA, 90 bp, synthetic construct
  source 1..90: mol_type = other DNA; note = MAGE_asnS
aggtggattataccgacgcagtgaccattctcgaaaactgcggcagaaagtttgaaaacccggtttactggggagtcgatctctcttctg

SEQ ID NO: 41 - DNA, 90 bp, synthetic construct
  source 1..90: mol_type = other DNA; note = MAGE_yceQ
taacaaggcttgcagtggaataatgaggccgtttccgtgtccattcttgttaaaacaagaaattttacggaataacccattttgcccgac

SEQ ID NO: 42 - DNA, 90 bp, synthetic construct
  source 1..90: mol_type = other DNA; note = MAGE_asd
gacatcaacatcaggcttacggtacagttaccgccaacaaaagttctgatgccattatttaatccgtcggtaatgacgtcctgattgacg

SEQ ID NO: 43 - DNA, 90 bp, synthetic construct
  source 1..90: mol_type = other DNA; note = MAGE_glyQ
cgagcccagtaatcctgtaaggtcaggatcaagccctggaaggttctggtatcaaacttttgcatattatttcgtgctggatacgtgtgg

SEQ ID NO: 44 - DNA, 90 bp, synthetic construct
  source 1..90: mol_type = other DNA; note = MAGE_folC
tcgtgcccactaaccgattctgaaacttacttgccaccgcttcttctcgcgtcaatcacttccatgacatgtgcgaccgtgtggaaagaa

SEQ ID NO: 45 - DNA, 33 bp, synthetic construct
  source 1..33: mol_type = other DNA; note = FlptFW
cttttgatcttcttctgtcaaaagttagtgagg

SEQ ID NO: 46 - DNA, 33 bp, synthetic construct
  source 1..33: mol_type = other DNA; note = FlptFMT
cttttgatcttcttctgtcaaaagttagtgaga

SEQ ID NO: 47 - DNA, 23 bp, synthetic construct
  source 1..23: mol_type = other DNA; note = RlptF
acaggcttaatggcaggataagc

SEQ ID NO: 48 - DNA, 22 bp, synthetic construct
  source 1..22: mol_type = other DNA; note = FdnaCW
ggcgatgaaagataccttcagg

SEQ ID NO: 49 - DNA, 22 bp, synthetic construct
  source 1..22: mol_type = other DNA; note = FdnaCMT
ggcgatgaaagataccttcaga

SEQ ID NO: 50 - DNA, 22 bp, synthetic construct
  source 1..22: mol_type = other DNA; note = RdnaC
tctttacctgttacccggctac

SEQ ID NO: 51 - DNA, 18 bp, synthetic construct
  source 1..18: mol_type = other DNA; note = FftsLW
catagccgggtggaaagg

SEQ ID NO: 52 - DNA, 18 bp, synthetic construct
  source 1..18: mol_type = other DNA; note = FftsLMT
catagccgggtggaaaga

SEQ ID NO: 53 - DNA, 19 bp, synthetic construct
  source 1..19: mol_type = other DNA; note = RtfsL
cagcgccaggagaatacag

SEQ ID NO: 54 - DNA, 28 bp, synthetic construct
  source 1..28: mol_type = other DNA; note = FlpxCW
gcgagataatacgatgatcaaacaaagg

SEQ ID NO: 55 - DNA, 28 bp, synthetic construct
  source 1..28: mol_type = other DNA; note = FlpxCMT
gcgagataatacgatgatcaaacaaaga

SEQ ID NO: 56 - DNA, 27 bp, synthetic construct
  source 1..27: mol_type = other DNA; note = RlpxC
catgaccggatttataagcggtaaatg

SEQ ID NO: 57 - DNA, 26 bp, synthetic construct
  source 1..26: mol_type = other DNA; note = FispUW
tggcccctgtagatttagtaattagg

SEQ ID NO: 58 - DNA, 26 bp, synthetic construct
  source 1..26: mol_type = other DNA; note = FispUMT
tggcccctgtagatttagtaattaga

SEQ ID NO: 59 - DNA, 22 bp, synthetic construct
  source 1..22: mol_type = other DNA; note = RispU
agaagggaacaatggttagcac

SEQ ID NO: 60 - DNA, 26 bp, synthetic construct
  source 1..26: mol_type = other DNA; note = FcdsAW
cttgcttgttgttactggtattcagg

SEQ ID NO: 61 - DNA, 26 bp, synthetic construct
  source 1..26: mol_type = other DNA; note = FcdsAMT
cttgcttgttgttactggtattcaga

SEQ ID NO: 62 - DNA, 21 bp, synthetic construct
  source 1..21: mol_type = other DNA; note = RcdsA
cgagtttggctgcacattttc

SEQ ID NO: 63 - DNA, 18 bp, synthetic construct
  source 1..18: mol_type = other DNA; note = FrsePW
ttgcaagcaggcgacagg

SEQ ID NO: 64 - DNA, 18 bp, synthetic construct
  source 1..18: mol_type = other DNA; note = FrsePMT
ttgcaagcaggcgacaga

SEQ ID NO: 65 - DNA, 20 bp, synthetic construct
  source 1..20: mol_type = other DNA; note = RrseP
tcgatcgcaaggaacagcag

SEQ ID NO: 66 - DNA, 17 bp, synthetic construct
  source 1..17: mol_type = other DNA; note = FtilSW
gcgacgcgttggtgagg

SEQ ID NO: 67 - DNA, 17 bp, synthetic construct
  source 1..17: mol_type = other DNA; note = FtilSMT
gcgacgcgttggtgaga

SEQ ID NO: 68 - DNA, 19 bp, synthetic construct
  source 1..19: mol_type = other DNA; note = RtilS
gcaatcagcgtttcgccat

SEQ ID NO: 69 - DNA, 20 bp, synthetic construct
  source 1..20: mol_type = other DNA; note = FmrdB
gctggacctcggtattgttc

SEQ ID NO: 70 - DNA, 26 bp, synthetic construct
  source 1..26: mol_type = other DNA; note = RmrdBW
gttacacgcttttcgacaacattttc

SEQ ID NO: 71 - DNA, 26 bp, synthetic construct
  source 1..26: mol_type = other DNA; note = RmrdBMT
gttacacgcttttcgacaacattttt

SEQ ID NO: 72 - DNA, 18 bp, synthetic construct
  source 1..18: mol_type = other DNA; note = FasnSW
ctcgaaaactgcggcagg

SEQ ID NO: 73 - DNA, 18 bp, synthetic construct
  source 1..18: mol_type = other DNA; note = FasnSMT
ctcgaaaactgcggcaga

SEQ ID NO: 74 - DNA, 22 bp, synthetic construct
  source 1..22: mol_type = other DNA; note = RasnS
accaagaccgaaacctgaatgc

SEQ ID NO: 75 - DNA, 19 bp, synthetic construct
  source 1..19: mol_type = other DNA; note = FyceQ
tgtcggttgcccgtttttc

SEQ ID NO: 76 - DNA, 18 bp, synthetic construct
  source 1..18: mol_type = other DNA; note = RyceQW
gccgtttccgtgtccatc

SEQ ID NO: 77 - DNA, 18 bp, synthetic construct
  source 1..18: mol_type = other DNA; note = RyceQMT
gccgtttccgtgtccatt

SEQ ID NO: 78 - DNA, 25 bp, synthetic construct
  source 1..25: mol_type = other DNA; note = FasDW
cgacggattaaataatggcatcagg

SEQ ID NO: 79 - DNA, 25 bp, synthetic construct
  source 1..25: mol_type = other DNA; note = FasDMT
cgacggattaaataatggcatcaga

SEQ ID NO: 80 - DNA, 21 bp, synthetic construct
  source 1..21: mol_type = other DNA; note = RasD
cgatcgttcggaacgactttc

SEQ ID NO: 81 - DNA, 32 bp, synthetic construct
  source 1..32: mol_type = other DNA; note = FglyQW
cacgaaataatatgcaaaagtttgataccagg

SEQ ID NO: 82 - DNA, 32 bp, synthetic construct
  source 1..32: mol_type = other DNA; note = FglyQMT
cacgaaataatatgcaaaagtttgataccaga

SEQ ID NO: 83 - DNA, 22 bp, synthetic construct
  source 1..22: mol_type = other DNA; note = RglyQ
cgaagttgtaagtggactgctc

SEQ ID NO: 84 - DNA, 24 bp, synthetic construct
  source 1..24: mol_type = other DNA; note = FfolC
tggaagtcagtgaaaatgccattc

SEQ ID NO: 85 - DNA, 20 bp, synthetic construct
  source 1..20: mol_type = other DNA; note = RfolCW
cttacttgccaccgcttctc

SEQ ID NO: 86 - DNA, 20 bp, synthetic construct
  source 1..20: mol_type = other DNA; note = RfolCMT
cttacttgccaccgcttctt

SEQ ID NO: 87 - DNA, 33 bp, synthetic construct
  source 1..33: mol_type = other DNA; note = FsgRNAvec
gttttagagctagaaatagcaagttaaaataag

SEQ ID NO: 88 - DNA, 26 bp, synthetic construct
  source 1..26: mol_type = other DNA; note = RsgRNAvec
gtgctcagtatctctatcactgatag

SEQ ID NO: 89 - DNA, 65 bp, synthetic construct
  source 1..65: mol_type = other DNA; note = sg_lptF1
cagtgatagagatactgagcactcttctgtcaaaagttagtggttttagagctagaaatagcaag

SEQ ID NO: 90 - DNA, 65 bp, synthetic construct
  source 1..65: mol_type = other DNA; note = sg_lptF2
cttgctatttctagctctaaaaccactaacttttgacagaagagtgctcagtatctctatcactg

SEQ ID NO: 91 - DNA, 65 bp, synthetic construct
  source 1..65: mol_type = other DNA; note = sg_dnaC1
cagtgatagagatactgagcaccggcgatgaaagataccttcgttttagagctagaaatagcaag

SEQ ID NO: 92 - DNA, 65 bp, synthetic construct
  source 1..65: mol_type = other DNA; note = sg_dnaC2
cttgctatttctagctctaaaacgaaggtatctttcatcgccggtgctcagtatctctatcactg

SEQ ID NO: 93 - DNA, 65 bp, synthetic construct
  source 1..65: mol_type = other DNA; note = sg_ftsL1
cagtgatagagatactgagcacgcgaccatagccgggtggaagttttagagctagaaatagcaag

SEQ ID NO: 94 - DNA, 65 bp, synthetic construct
  source 1..65: mol_type = other DNA; note = sg_ftsL2
cttgctatttctagctctaaaacttccacccggctatggtcgcgtgctcagtatctctatcactg

SEQ ID NO: 95 - DNA, 65 bp, synthetic construct
  source 1..65: mol_type = other DNA; note = sg_lpxC1
cagtgatagagatactgagcacataatacgatgatcaaacaagttttagagctagaaatagcaag

SEQ ID NO: 96 - DNA, 65 bp, synthetic construct
  source 1..65: mol_type = other DNA; note = sg_lpxC2
cttgctatttctagctctaaaacttgtttgatcatcgtattatgtgctcagtatctctatcactg

SEQ ID NO: 97 - DNA, 65 bp, synthetic construct
  source 1..65: mol_type = other DNA; note = sg_ispU1
cagtgatagagatactgagcaccccctgtagatttagtaattgttttagagctagaaatagcaag

SEQ ID NO: 98 - DNA, 65 bp, synthetic construct
  source 1..65: mol_type = other DNA; note = sg_ispU2
cttgctatttctagctctaaaacaattactaaatctacagggggtgctcagtatctctatcactg

SEQ ID NO: 99 - DNA, 65 bp, synthetic construct
  source 1..65: mol_type = other DNA; note = sg_cdsA1
cagtgatagagatactgagcacgcttgttgttactggtattcgttttagagctagaaatagcaag

SEQ ID NO: 100 - DNA, 65 bp, synthetic construct
  source 1..65: mol_type = other DNA; note = sg_cdsA2
cttgctatttctagctctaaaacgaataccagtaacaacaagcgtgctcagtatctctatcactg

SEQ ID NO: 101 - DNA, 65 bp, synthetic construct
  source 1..65: mol_type = other DNA; note = sg_rseP1
cagtgatagagatactgagcaccaggtttgcaagcaggcgacgttttagagctagaaatagcaag

SEQ ID NO: 102 - DNA, 65 bp, synthetic construct
  source 1..65: mol_type = other DNA; note = sg_rseP2
cttgctatttctagctctaaaacgtcgcctgcttgcaaacctggtgctcagtatctctatcactg

SEQ ID NO: 103 - DNA, 65 bp, synthetic construct
  source 1..65: mol_type = other DNA; note = sg_tilS1
cagtgatagagatactgagcaccttcccgcgacgcgttggtggttttagagctagaaatagcaag

SEQ ID NO: 104 - DNA, 65 bp, synthetic construct
  source 1..65: mol_type = other DNA; note = sg_tilS2
cttgctatttctagctctaaaaccaccaacgcgtcgcgggaaggtgctcagtatctctatcactg

SEQ ID NO: 105 - DNA, 65 bp, synthetic construct
  source 1..65: mol_type = other DNA; note = sg_mrdB1
cagtgatagagatactgagcactaatgtcaatccacacccacgttttagagctagaaatagcaag

SEQ ID NO: 106 - DNA, 65 bp, synthetic construct
  source 1..65: mol_type = other DNA; note = sg_mrdB2
cttgctatttctagctctaaaacgtgggtgtggattgacattagtgctcagtatctctatcactg

SEQ ID NO: 107 - DNA, 65 bp, synthetic construct
  source 1..65: mol_type = other DNA; note = sg_asnS1
cagtgatagagatactgagcacccattctcgaaaactgcggcgttttagagctagaaatagcaag

SEQ ID NO: 108 - DNA, 65 bp, synthetic construct
  source 1..65: mol_type = other DNA; note = sg_asnS2
cttgctatttctagctctaaaacgccgcagttttcgagaatgggtgctcagtatctctatcactg

SEQ ID NO: 109 - DNA, 65 bp, synthetic construct
  source 1..65: mol_type = other DNA; note = sg_yceQ1
cagtgatagagatactgagcactaaaatttcttgttttaacagttttagagctagaaatagcaag

SEQ ID NO: 110 - DNA, 65 bp, synthetic construct
  source 1..65: mol_type = other DNA; note = sg_yceQ2
cttgctatttctagctctaaaactgttaaaacaagaaattttagtgctcagtatctctatcactg

SEQ ID NO: 111 - DNA, 65 bp, synthetic construct
  source 1..65: mol_type = other DNA; note = sg_asD1
cagtgatagagatactgagcacacggattaaataatggcatcgttttagagctagaaatagcaag

SEQ ID NO: 112 - DNA, 65 bp, synthetic construct
  source 1..65: mol_type = other DNA; note = sg_asD2
cttgctatttctagctctaaaacgatgccattatttaatccgtgtgctcagtatctctatcactg

SEQ ID NO: 113 - DNA, 65 bp, synthetic construct
  source 1..65: mol_type = other DNA; note = sg_glyQ1
cagtgatagagatactgagcacatatgcaaaagtttgataccgttttagagctagaaatagcaag

SEQ ID NO: 114 - DNA, 65 bp, synthetic construct
  source 1..65: mol_type = other DNA; note = sg_glyQ2
cttgctatttctagctctaaaacggtatcaaacttttgcatatgtgctcagtatctctatcactg

SEQ ID NO: 115 - DNA, 65 bp, synthetic construct
  source 1..65: mol_type = other DNA; note = sg_folC1
cagtgatagagatactgagcactcatggaagtgattgacgcggttttagagctagaaatagcaag

SEQ ID NO: 116 - DNA, 65 bp, synthetic construct
  source 1..65: mol_type = other DNA; note = sg_folC2
cttgctatttctagctctaaaaccgcgtcaatcacttccatgagtgctcagtatctctatcactg